European Patent Specification EP 3 698 142 B1, published April 30, 2025. Title: Type XVI Collagen Assay. Applicant: Nordic Bioscience A/S. The sequence listing filed with the application follows.

SEQUENCE LISTING (7 sequences)

SEQ ID NO: 1 - protein, 10 aa, Artificial Sequence
  C-terminus biomarker
PMKTMKGPFG

SEQ ID NO: 2 - protein, 11 aa, Artificial Sequence
  elongated peptide
PMKTMKGPFGG

SEQ ID NO: 3 - protein, 9 aa, Artificial Sequence
  Truncated peptide
PMKTMKGPF

SEQ ID NO: 4 - protein, 10 aa, Artificial Sequence
  SITE 1: Biotinylated, with optional linker between biotin and peptide
  Biotinylated peptide with optional linker
PMKTMKGPFG

SEQ ID NO: 5 - protein, 10 aa, Artificial Sequence
  nonsense peptide
VPKDLPPDTT

SEQ ID NO: 6 - protein, 10 aa, Artificial Sequence
  SITE 1: Biotinylated, with optional linker between peptide and biotin
  biotinylated nonsense peptide
VPKDLPPDTT

SEQ ID NO: 7 - protein, 13 aa, Artificial Sequence
  SITE 1: KLH attached
  immunogenic peptide
CGGPMKTMKGPFG